European Patent Specification EP 3 696 266 B1, published April 3, 2024. Title: Use of pluripotent cells having modified differentiation potential in the preparation of somatic chimera aminals. Applicant: The University of Tokyo. The sequence listing filed with the application follows.

SEQUENCE LISTING (9 sequences)

SEQ ID NO: 1 - DNA, 20 bp, Artificial Sequence
  gRNA-1 targeting Prdm14
gaacctcgccaccaccgagg

SEQ ID NO: 2 - DNA, 20 bp, Artificial Sequence
  gRNA-2 targeting Prdm14
gtatggagccatcgctagtc

SEQ ID NO: 3 - DNA, 31 bp, Artificial Sequence
  Example of knocked out Prdm14
ctcgccaccaccggtccggagcacccaaccg

SEQ ID NO: 4 - DNA, 34 bp, Artificial Sequence
  Example 2 of knocked out Prdm14
ctcgccaccaccgcagtattaaaacatggatgta

SEQ ID NO: 5 - DNA, 20 bp, Artificial Sequence
  Otx2 targeting sequence in gRNA1
gagtctgaccacttcgggta

SEQ ID NO: 6 - DNA, 20 bp, Artificial Sequence
  Otx2 targeting sequence in gRNA2
gtatggagccatcgctagtc

SEQ ID NO: 7 - DNA, 21 bp, Artificial Sequence
  Forward primer for Pdx1 amplification
attgagatgagaaccggcatg

SEQ ID NO: 8 - DNA, 21 bp, Artificial Sequence
  Reverse primer for WT Pdx1 amplification
ttcatgcgacggttttggaac

SEQ ID NO: 9 - DNA, 18 bp, Artificial Sequence
  Reverse primer for mutant Pdx1 amplification
tgtgagcgagtaacaacc